European Patent Specification EP 4 048 808 B1, published December 11, 2024. Title: METHYLATION DETECTION AND ANALYSIS OF MAMMALIAN DNA. Applicant: Peking University. The sequence listing filed with the application follows.

SEQUENCE LISTING (43 sequences)

SEQ ID NO: 1 - DNA, 19 bp, artificial sequence
  one strand of Nextera transposon
ctgtctcttatacacatct

SEQ ID NO: 2 - DNA, 33 bp, artificial sequence
  one 5mC modified strand of Nextera transposon P5
  modified_base (2)..(2): n is methylated cytosine
  modified_base (5)..(5): n is methylated cytosine
  modified_base (8)..(8): n is methylated cytosine
  modified_base (11)..(11): n is methylated cytosine
  modified_base (14)..(14): n is methylated cytosine
  modified_base (31)..(31): n is methylated cytosine
tngtnggnagngtnagatgtgtataagaganag

SEQ ID NO: 3 - DNA, 34 bp, artificial sequence
  one 5mC modified strand of Nextera transposon P7
  modified_base (3)..(3): n is methylated cytosine
  modified_base (5)..(5): n is methylated cytosine
  modified_base (11)..(11): n is methylated cytosine
  modified_base (13)..(13): n is methylated cytosine
  modified_base (32)..(32): n is methylated cytosine
gtntngtgggntnggagatgtgtataagaganag

SEQ ID NO: 4 - DNA, 47 bp, artificial sequence
  Nextera index primer
caagcagaagacggcatacgagattcgccttagtctcgtgggctcgg

SEQ ID NO: 5 - DNA, 47 bp, artificial sequence
  Nextera index primer
caagcagaagacggcatacgagatctagtacggtctcgtgggctcgg

SEQ ID NO: 6 - DNA, 47 bp, artificial sequence
  Nextera index primer
caagcagaagacggcatacgagatttctgcctgtctcgtgggctcgg

SEQ ID NO: 7 - DNA, 47 bp, artificial sequence
  Nextera index primer
caagcagaagacggcatacgagatgctcaggagtctcgtgggctcgg

SEQ ID NO: 8 - DNA, 47 bp, artificial sequence
  Nextera index primer
caagcagaagacggcatacgagataggagtccgtctcgtgggctcgg

SEQ ID NO: 9 - DNA, 47 bp, artificial sequence
  Nextera index primer
caagcagaagacggcatacgagatcatgcctagtctcgtgggctcgg

SEQ ID NO: 10 - DNA, 47 bp, artificial sequence
  Nextera index primer
caagcagaagacggcatacgagatgtagagaggtctcgtgggctcgg

SEQ ID NO: 11 - DNA, 47 bp, artificial sequence
  Nextera index primer
caagcagaagacggcatacgagatcctctctggtctcgtgggctcgg

SEQ ID NO: 12 - DNA, 47 bp, artificial sequence
  Nextera index primer
caagcagaagacggcatacgagatagcgtagcgtctcgtgggctcgg

SEQ ID NO: 13 - DNA, 47 bp, artificial sequence
  Nextera index primer
caagcagaagacggcatacgagatcagcctcggtctcgtgggctcgg

SEQ ID NO: 14 - DNA, 47 bp, artificial sequence
  Nextera index primer
caagcagaagacggcatacgagattgcctcttgtctcgtgggctcgg

SEQ ID NO: 15 - DNA, 47 bp, artificial sequence
  Nextera index primer
caagcagaagacggcatacgagattcctctacgtctcgtgggctcgg

SEQ ID NO: 16 - DNA, 51 bp, artificial sequence
  Nextera index primer
aatgatacggcgaccaccgagatctacactagatcgctcgtcggcagcgtc

SEQ ID NO: 17 - DNA, 51 bp, artificial sequence
  Nextera index primer
aatgatacggcgaccaccgagatctacacctctctattcgtcggcagcgtc

SEQ ID NO: 18 - DNA, 51 bp, artificial sequence
  Nextera index primer
aatgatacggcgaccaccgagatctacactatcctcttcgtcggcagcgtc

SEQ ID NO: 19 - DNA, 51 bp, artificial sequence
  Nextera index primer
aatgatacggcgaccaccgagatctacacagagtagatcgtcggcagcgtc

SEQ ID NO: 20 - DNA, 51 bp, artificial sequence
  Nextera index primer
aatgatacggcgaccaccgagatctacacgtaaggagtcgtcggcagcgtc

SEQ ID NO: 21 - DNA, 51 bp, artificial sequence
  Nextera index primer
aatgatacggcgaccaccgagatctacacactgcatatcgtcggcagcgtc

SEQ ID NO: 22 - DNA, 51 bp, artificial sequence
  Nextera index primer
aatgatacggcgaccaccgagatctacacaaggagtatcgtcggcagcgtc

SEQ ID NO: 23 - DNA, 51 bp, artificial sequence
  Nextera index primer
aatgatacggcgaccaccgagatctacacctaagccttcgtcggcagcgtc

SEQ ID NO: 24 - DNA, 20 bp, artificial sequence
  transposon primer binding site sequence
  modified_base (6)..(7): n is methylated cytosine
  modified_base (13)..(14): n is methylated cytosine
  modified_base (18)..(18): n is methylated cytosine
agaagnngtgtgnnggtnta

SEQ ID NO: 25 - DNA, 20 bp, artificial sequence
  transposon primer binding site sequence
  modified_base (3)..(3): n is methylated cytosine
  modified_base (7)..(7): n is methylated cytosine
  modified_base (11)..(11): n is methylated cytosine
  modified_base (16)..(16): n is methylated cytosine
  modified_base (19)..(19): n is methylated cytosine
atngtgnggangaganagna

SEQ ID NO: 26 - DNA, 20 bp, artificial sequence
  transposon primer binding site sequence
  modified_base (4)..(5): n is methylated cytosine
  modified_base (9)..(9): n is methylated cytosine
  modified_base (11)..(12): n is methylated cytosine
  modified_base (17)..(17): n is methylated cytosine
  modified_base (19)..(20): n is methylated cytosine
aatnntagnannggttngnn

SEQ ID NO: 27 - DNA, 20 bp, artificial sequence
  transposon primer binding site sequence
  modified_base (2)..(2): n is methylated cytosine
  modified_base (9)..(9): n is methylated cytosine
  modified_base (15)..(15): n is methylated cytosine
  modified_base (17)..(17): n is methylated cytosine
  modified_base (19)..(19): n is methylated cytosine
angtgttgnaggtgnantng

SEQ ID NO: 28 - DNA, 20 bp, artificial sequence
  transposon primer binding site sequence
  modified_base (2)..(2): n is methylated cytosine
  modified_base (4)..(5): n is methylated cytosine
  modified_base (7)..(7): n is methylated cytosine
  modified_base (9)..(9): n is methylated cytosine
  modified_base (12)..(13): n is methylated cytosine
  modified_base (20)..(20): n is methylated cytosine
anannananggnntagagtn

SEQ ID NO: 29 - DNA, 20 bp, artificial sequence
  transposon primer binding site sequence
  modified_base (5)..(5): n is methylated cytosine
  modified_base (9)..(9): n is methylated cytosine
  modified_base (11)..(11): n is methylated cytosine
  modified_base (13)..(13): n is methylated cytosine
  modified_base (16)..(17): n is methylated cytosine
  modified_base (20)..(20): n is methylated cytosine
tgganaatnangngannagn

SEQ ID NO: 30 - DNA, 20 bp, artificial sequence
  transposon primer binding site sequence
  modified_base (2)..(2): n is methylated cytosine
  modified_base (5)..(5): n is methylated cytosine
  modified_base (9)..(9): n is methylated cytosine
  modified_base (11)..(11): n is methylated cytosine
  modified_base (13)..(13): n is methylated cytosine
  modified_base (15)..(16): n is methylated cytosine
  modified_base (20)..(20): n is methylated cytosine
tnatntaangngnanngtgn

SEQ ID NO: 31 - DNA, 20 bp, artificial sequence
  transposon primer binding site sequence
  modified_base (3)..(3): n is methylated cytosine
  modified_base (6)..(6): n is methylated cytosine
  modified_base (9)..(9): n is methylated cytosine
  modified_base (11)..(11): n is methylated cytosine
  modified_base (13)..(13): n is methylated cytosine
  modified_base (15)..(15): n is methylated cytosine
  modified_base (19)..(20): n is methylated cytosine
ttngtnggntntntngaann

SEQ ID NO: 32 - DNA, 20 bp, artificial sequence
  transposon primer binding site sequence
  modified_base (9)..(9): n is methylated cytosine
  modified_base (13)..(13): n is methylated cytosine
  modified_base (17)..(17): n is methylated cytosine
  modified_base (19)..(19): n is methylated cytosine
tggtggagngtgnagantnt

SEQ ID NO: 33 - DNA, 20 bp, artificial sequence
  transposon primer binding site sequence
  modified_base (4)..(4): n is methylated cytosine
  modified_base (7)..(8): n is methylated cytosine
  modified_base (11)..(11): n is methylated cytosine
  modified_base (13)..(13): n is methylated cytosine
  modified_base (16)..(16): n is methylated cytosine
  modified_base (20)..(20): n is methylated cytosine
tatnttnntgngnagnggan

SEQ ID NO: 34 - DNA, 20 bp, artificial sequence
  transposon primer binding site sequence
  modified_base (1)..(1): n is methylated cytosine
  modified_base (5)..(5): n is methylated cytosine
  modified_base (14)..(14): n is methylated cytosine
  modified_base (16)..(16): n is methylated cytosine
ntgangtgtgaggngntaga

SEQ ID NO: 35 - DNA, 20 bp, artificial sequence
  transposon primer binding site sequence
  modified_base (1)..(2): n is methylated cytosine
  modified_base (5)..(5): n is methylated cytosine
  modified_base (8)..(9): n is methylated cytosine
  modified_base (12)..(13): n is methylated cytosine
  modified_base (16)..(16): n is methylated cytosine
  modified_base (19)..(19): n is methylated cytosine
nnatnatnnaannggnttng

SEQ ID NO: 36 - DNA, 20 bp, artificial sequence
  transposon primer binding site sequence
  modified_base (1)..(1): n is methylated cytosine
  modified_base (3)..(3): n is methylated cytosine
  modified_base (10)..(11): n is methylated cytosine
  modified_base (14)..(15): n is methylated cytosine
  modified_base (17)..(17): n is methylated cytosine
nangagaagnngtnngntta

SEQ ID NO: 37 - DNA, 20 bp, artificial sequence
  transposon primer binding site sequence
  modified_base (1)..(1): n is methylated cytosine
  modified_base (5)..(5): n is methylated cytosine
  modified_base (9)..(9): n is methylated cytosine
  modified_base (12)..(12): n is methylated cytosine
  modified_base (14)..(14): n is methylated cytosine
  modified_base (16)..(17): n is methylated cytosine
  modified_base (19)..(19): n is methylated cytosine
ngtangtgnaanantnngnt

SEQ ID NO: 38 - DNA, 20 bp, artificial sequence
  transposon primer binding site sequence
  modified_base (1)..(1): n is methylated cytosine
  modified_base (7)..(7): n is methylated cytosine
  modified_base (11)..(11): n is methylated cytosine
  modified_base (18)..(18): n is methylated cytosine
  modified_base (20)..(20): n is methylated cytosine
nttggtnaggngagaagnan

SEQ ID NO: 39 - DNA, 20 bp, artificial sequence
  transposon primer binding site sequence
  modified_base (3)..(3): n is methylated cytosine
  modified_base (9)..(9): n is methylated cytosine
  modified_base (14)..(14): n is methylated cytosine
ggngtgatnagtgngtggat

SEQ ID NO: 40 - DNA, 20 bp, artificial sequence
  transposon primer binding site sequence
  modified_base (4)..(4): n is methylated cytosine
  modified_base (14)..(15): n is methylated cytosine
  modified_base (17)..(18): n is methylated cytosine
gagngtttggtganngnnat

SEQ ID NO: 41 - DNA, 20 bp, artificial sequence
  transposon primer binding site sequence
  modified_base (2)..(3): n is methylated cytosine
  modified_base (6)..(6): n is methylated cytosine
  modified_base (10)..(11): n is methylated cytosine
  modified_base (17)..(18): n is methylated cytosine
gnntgnggtnnattgannta

SEQ ID NO: 42 - DNA, 20 bp, artificial sequence
  transposon primer binding site sequence
  modified_base (6)..(7): n is methylated cytosine
  modified_base (9)..(9): n is methylated cytosine
  modified_base (11)..(12): n is methylated cytosine
  modified_base (15)..(15): n is methylated cytosine
  modified_base (18)..(18): n is methylated cytosine
  modified_base (20)..(20): n is methylated cytosine
gtaagnnantnnagngtnan

SEQ ID NO: 43 - DNA, 20 bp, artificial sequence
  transposon primer binding site sequence
  modified_base (4)..(4): n is methylated cytosine
  modified_base (10)..(10): n is methylated cytosine
  modified_base (12)..(12): n is methylated cytosine
  modified_base (15)..(15): n is methylated cytosine
gatntgttgngngtntggtg